European Patent Application EP 4 653 460 A1, published November 26, 2025. Title: IL18R AGONIST ANTIBODIES AND USES THEREOF. Applicant: Egle Therapeutics. Application EP. The sequence listing filed with the application follows.

SEQUENCE LISTING (8 sequences)

SEQ ID NO: 1 - protein, 9 aa, synthetic construct
GYSITSGYY

SEQ ID NO: 2 - protein, 7 aa, synthetic construct
ITYDGIN

SEQ ID NO: 3 - protein, 13 aa, synthetic construct
CATPYYGTSGFAY

SEQ ID NO: 4 - protein, 119 aa, synthetic construct
DVQLQESGPGLVKFFQSLSLTCSVTGYSITSGYYWNWVRQFPGNKLEWLGYITYDGINDYNPSLKNRISITRDTSKNQFFLRLNSVTTEDTATYYCATPYYGTSGFAYWGQGTLVTVSA

SEQ ID NO: 5 - protein, 5 aa, synthetic construct
SSVGY

SEQ ID NO: 6 - skipped

SEQ ID NO: 7 - protein, 9 aa, synthetic construct
QQWSSIPLT

SEQ ID NO: 8 - protein, 106 aa, synthetic construct
QIVLTQSPAIMSASPGEKVTMTCSASSSVGYMHWYQQRSGTSPKRWIYDTSKLPSGVPARFSASGSGTSYSLTISSMESEDAATYYCQQWSSIPLTFGAGTKLELK